European Patent Application EP 4 491 744 A1, published January 15, 2025. Title: PRIMER SET, KIT FOR DETERMINING WHETHER OR NOT SUBJECT HAS DEVELOPED SPINAL MUSCULAR ATROPHY AND/OR RISK OF DEVELOPING SPINAL MUSCULAR ATROPHY, AND METHOD FOR DETERMINING WHETHER OR NOT SUBJECT HAS DEVELOPED SPINAL MUSCULAR ATROPHY AND/OR RISK OF DEVELOPING SPINAL MUSCULAR ATROPHY. Applicant: CRAIF INC. Application WO. The sequence listing filed with the application follows.

SEQUENCE LISTING (81 sequences)

SEQ ID NO: 1 - DNA, 1135 bp, Homo sapiens
  source 1..1135: mol_type = genomic DNA
aattgttttctttgggataacttttaaagtacattaaaagactatcaacttaatttctgatcatattttgttgaataaaataagtaaaatgtcttgtgaaacaaaatgctttttaacatccatataaagctatctatatatagctatctatgtctatatagctattttttttaacttcctttattttccttacagggtttcagacaaaatcaaaaagaaggaaggtgctcacattccttaaattaaggagtaagtctgccagcattatgaaagtgaatcttacttttgtaaaactttatggtttgtggaaaacaaatgtttttgaacatttaaaaagttcagatgttaaaaagttgaaaggttaatgtaaaacaatcaatattaaagaattttgatgccaaaactattagataaaaggttaatctacatccctactagaattctcatacttaactggttggttatgtggaagaaacatactttcacaataaagagctttaggatatgatgccattttatatcactagtaggcagaccagcagacttttttttattgtgatatgggataacctaggcatactgcactgtacactctgacatatgaagtgctctagtcaagtttaactggtgtccacagaggacatggtttaactggaattcgtcaagcctctggttctaatttctcatttgcaggaaatgctggcatagagcagcactaaatgacaccactaaagaaacgatcagacagatctggaatgtgaagcgttatagaagataactggcctcatttcttcaaaatatcaagtgttgggaaagaaaaaaggaagtggaatgggtaactcttcttgattaaaagttatgtaataaccaaatgcaatgtgaaatattttactggactctattttgaaaaaccatctgtaaaagactggggtgggggtgggaggccagcacggtggtgaggcagttgagaaaatttgaatgtggattagattttgaatgatattggataattattggtaattttatgagctgtgagaagggtgttgtagtttataaaagactgtcttaatttgcatacttaagcatttaggaatgaagtgttagagtgtcttaaaatgtttcaaatggtttaaca

SEQ ID NO: 2 - DNA, 1135 bp, Homo sapiens
  source 1..1135: mol_type = genomic DNA
aattgttttctttgggataacttttaaagtacattaaaagactatcaacttaatttctgatcatattttgttgaataaaataagtaaaatgtcttgtgaaacaaaatgctttttaacatccatataaagctatctatatatagctatctatatctatatagctattttttttaacttcctttattttccttacagggttttagacaaaatcaaaaagaaggaaggtgctcacattccttaaattaaggagtaagtctgccagcattatgaaagtgaatcttacttttgtaaaactttatggtttgtggaaaacaaatgtttttgaacatttaaaaagttcagatgttagaaagttgaaaggttaatgtaaaacaatcaatattaaagaattttgatgccaaaactattagataaaaggttaatctacatccctactagaattctcatacttaactggttggttgtgtggaagaaacatactttcacaataaagagctttaggatatgatgccattttatatcactagtaggcagaccagcagacttttttttattgtgatatgggataacctaggcatactgcactgtacactctgacatatgaagtgctctagtcaagtttaactggtgtccacagaggacatggtttaactggaattcgtcaagcctctggttctaatttctcatttgcaggaaatgctggcatagagcagcactaaatgacaccactaaagaaacgatcagacagatctggaatgtgaagcgttatagaagataactggcctcatttcttcaaaatatcaagtgttgggaaagaaaaaaggaagtggaatgggtaactcttcttgattaaaagttatgtaataaccaaatgcaatgtgaaatattttactggactctattttgaaaaaccatctgtaaaagactgaggtgggggtgggaggccagcacggtggtgaggcagttgagaaaatttgaatgtggattagattttgaatgatattggataattattggtaattttatgagctgtgagaagggtgttgtagtttataaaagactgtcttaatttgcatacttaagcatttaggaatgaagtgttagagtgtcttaaaatgtttcaaatggtttaaca

SEQ ID NO: 3 - DNA, 22 bp, synthetic construct
  source 1..22: mol_type = other DNA
tatctatatatagctatctatg

SEQ ID NO: 4 - DNA, 22 bp, synthetic construct
  source 1..22: mol_type = other DNA
atctatatatagctatctatgt

SEQ ID NO: 5 - DNA, 22 bp, synthetic construct
  source 1..22: mol_type = other DNA
tctatatatagctatctatgtc

SEQ ID NO: 6 - DNA, 22 bp, synthetic construct
  source 1..22: mol_type = other DNA
ctatatatagctatctatgtct

SEQ ID NO: 7 - DNA, 22 bp, synthetic construct
  source 1..22: mol_type = other DNA
tttattttccttacagggtttc

SEQ ID NO: 8 - DNA, 22 bp, synthetic construct
  source 1..22: mol_type = other DNA
ttattttccttacagggtttca

SEQ ID NO: 9 - DNA, 22 bp, synthetic construct
  source 1..22: mol_type = other DNA
tattttccttacagggtttcag

SEQ ID NO: 10 - DNA, 22 bp, synthetic construct
  source 1..22: mol_type = other DNA
attttccttacagggtttcaga

SEQ ID NO: 11 - DNA, 22 bp, synthetic construct
  source 1..22: mol_type = other DNA
atttaaaaagttcagatgttaa

SEQ ID NO: 12 - DNA, 22 bp, synthetic construct
  source 1..22: mol_type = other DNA
tttaaaaagttcagatgttaaa

SEQ ID NO: 13 - DNA, 22 bp, synthetic construct
  source 1..22: mol_type = other DNA
ttaaaaagttcagatgttaaaa

SEQ ID NO: 14 - DNA, 22 bp, synthetic construct
  source 1..22: mol_type = other DNA
taaaaagttcagatgttaaaaa

SEQ ID NO: 15 - DNA, 22 bp, synthetic construct
  source 1..22: mol_type = other DNA
ctcatacttaactggttggtta

SEQ ID NO: 16 - DNA, 22 bp, synthetic construct
  source 1..22: mol_type = other DNA
tcatacttaactggttggttat

SEQ ID NO: 17 - DNA, 22 bp, synthetic construct
  source 1..22: mol_type = other DNA
catacttaactggttggttatg

SEQ ID NO: 18 - DNA, 22 bp, synthetic construct
  source 1..22: mol_type = other DNA
atacttaactggttggttatgt

SEQ ID NO: 19 - DNA, 22 bp, synthetic construct
  source 1..22: mol_type = other DNA
tccttctttttgattttgtctg

SEQ ID NO: 20 - DNA, 22 bp, synthetic construct
  source 1..22: mol_type = other DNA
ccttctttttgattttgtctga

SEQ ID NO: 21 - DNA, 22 bp, synthetic construct
  source 1..22: mol_type = other DNA
cttctttttgattttgtctgaa

SEQ ID NO: 22 - DNA, 22 bp, synthetic construct
  source 1..22: mol_type = other DNA
ttctttttgattttgtctgaaa

SEQ ID NO: 23 - DNA, 22 bp, synthetic construct
  source 1..22: mol_type = other DNA
ttacattaacctttcaactttt

SEQ ID NO: 24 - DNA, 22 bp, synthetic construct
  source 1..22: mol_type = other DNA
tacattaacctttcaacttttt

SEQ ID NO: 25 - DNA, 22 bp, synthetic construct
  source 1..22: mol_type = other DNA
acattaacctttcaactttttc

SEQ ID NO: 26 - DNA, 22 bp, synthetic construct
  source 1..22: mol_type = other DNA
cattaacctttcaactttttcc

SEQ ID NO: 27 - DNA, 22 bp, synthetic construct
  source 1..22: mol_type = other DNA
tgaaagtatgtttcttccacat

SEQ ID NO: 28 - DNA, 22 bp, synthetic construct
  source 1..22: mol_type = other DNA
gaaagtatgtttcttccacata

SEQ ID NO: 29 - DNA, 22 bp, synthetic construct
  source 1..22: mol_type = other DNA
aaagtatgtttcttccacataa

SEQ ID NO: 30 - DNA, 22 bp, synthetic construct
  source 1..22: mol_type = other DNA
aagtatgtttcttccacataac

SEQ ID NO: 31 - DNA, 22 bp, synthetic construct
  source 1..22: mol_type = other DNA
tgctggcctcccacccccaccc

SEQ ID NO: 32 - DNA, 22 bp, synthetic construct
  source 1..22: mol_type = other DNA
gctggcctcccacccccacccc

SEQ ID NO: 33 - DNA, 22 bp, synthetic construct
  source 1..22: mol_type = other DNA
ctggcctcccacccccacccca

SEQ ID NO: 34 - DNA, 22 bp, synthetic construct
  source 1..22: mol_type = other DNA
tggcctcccacccccaccccag

SEQ ID NO: 35 - DNA, 30 bp, synthetic construct
  source 1..30: mol_type = other DNA
acttcctttattttccttacagggttccag

SEQ ID NO: 36 - DNA, 29 bp, synthetic construct
  source 1..29: mol_type = other DNA
cttcctttattttccttacagggttccag

SEQ ID NO: 37 - DNA, 28 bp, synthetic construct
  source 1..28: mol_type = other DNA
ttcctttattttccttacagggttccag

SEQ ID NO: 38 - DNA, 27 bp, synthetic construct
  source 1..27: mol_type = other DNA
tcctttattttccttacagggttccag

SEQ ID NO: 39 - DNA, 26 bp, synthetic construct
  source 1..26: mol_type = other DNA
cctttattttccttacagggttccag

SEQ ID NO: 40 - DNA, 25 bp, synthetic construct
  source 1..25: mol_type = other DNA
ctttattttccttacagggttccag

SEQ ID NO: 41 - DNA, 24 bp, synthetic construct
  source 1..24: mol_type = other DNA
tttattttccttacagggttccag

SEQ ID NO: 42 - DNA, 30 bp, synthetic construct
  source 1..30: mol_type = other DNA
ggattgttttacattaacctttcaactttt

SEQ ID NO: 43 - DNA, 29 bp, synthetic construct
  source 1..29: mol_type = other DNA
gattgttttacattaacctttcaactttt

SEQ ID NO: 44 - DNA, 28 bp, synthetic construct
  source 1..28: mol_type = other DNA
attgttttacattaacctttcaactttt

SEQ ID NO: 45 - DNA, 27 bp, synthetic construct
  source 1..27: mol_type = other DNA
ttgttttacattaacctttcaactttt

SEQ ID NO: 46 - DNA, 26 bp, synthetic construct
  source 1..26: mol_type = other DNA
tgttttacattaacctttcaactttt

SEQ ID NO: 47 - DNA, 25 bp, synthetic construct
  source 1..25: mol_type = other DNA
gttttacattaacctttcaactttt

SEQ ID NO: 48 - DNA, 24 bp, synthetic construct
  source 1..24: mol_type = other DNA
ttttacattaacctttcaactttt

SEQ ID NO: 49 - DNA, 28 bp, synthetic construct
  source 1..28: mol_type = other DNA
cttcctttattttccttacagggttcca

SEQ ID NO: 50 - DNA, 28 bp, synthetic construct
  source 1..28: mol_type = other DNA
acttcctttattttccttacagggttcc

SEQ ID NO: 51 - DNA, 28 bp, synthetic construct
  source 1..28: mol_type = other DNA
ttcctttattttccttacagggtttcag

SEQ ID NO: 52 - DNA, 28 bp, synthetic construct
  source 1..28: mol_type = other DNA
cttcctttattttccttacagggtttca

SEQ ID NO: 53 - DNA, 28 bp, synthetic construct
  source 1..28: mol_type = other DNA
acttcctttattttccttacagggtttc

SEQ ID NO: 54 - DNA, 28 bp, synthetic construct
  source 1..28: mol_type = other DNA
tcctttattttccttacagggtttccga

SEQ ID NO: 55 - DNA, 28 bp, synthetic construct
  source 1..28: mol_type = other DNA
ttcctttattttccttacagggtttccg

SEQ ID NO: 56 - DNA, 28 bp, synthetic construct
  source 1..28: mol_type = other DNA
cttcctttattttccttacagggtttcc

SEQ ID NO: 57 - DNA, 27 bp, synthetic construct
  source 1..27: mol_type = other DNA
tgttttacattaacctttcaacttttt

SEQ ID NO: 58 - DNA, 27 bp, synthetic construct
  source 1..27: mol_type = other DNA
gttttacattaacctttcaacttttta

SEQ ID NO: 59 - DNA, 27 bp, synthetic construct
  source 1..27: mol_type = other DNA
tgttttacattaacctttcaactttta

SEQ ID NO: 60 - DNA, 27 bp, synthetic construct
  source 1..27: mol_type = other DNA
ttgttttacattaacctttcaacttct

SEQ ID NO: 61 - DNA, 27 bp, synthetic construct
  source 1..27: mol_type = other DNA
tgttttacattaacctttcaacttctt

SEQ ID NO: 62 - DNA, 27 bp, synthetic construct
  source 1..27: mol_type = other DNA
gttttacattaacctttcaacttctta

SEQ ID NO: 63 - DNA, 24 bp, synthetic construct
  source 1..24: mol_type = other DNA
gtgaaagtatgtttcttccacata

SEQ ID NO: 64 - DNA, 25 bp, synthetic construct
  source 1..25: mol_type = other DNA
tgtgaaagtatgtttcttccacata

SEQ ID NO: 65 - DNA, 26 bp, synthetic construct
  source 1..26: mol_type = other DNA
ttgtgaaagtatgtttcttccacata

SEQ ID NO: 66 - DNA, 24 bp, synthetic construct
  source 1..24: mol_type = other DNA
tgtgaaagtatgtttcttccacat

SEQ ID NO: 67 - DNA, 25 bp, synthetic construct
  source 1..25: mol_type = other DNA
ttgtgaaagtatgtttcttccacat

SEQ ID NO: 68 - DNA, 26 bp, synthetic construct
  source 1..26: mol_type = other DNA
attgtgaaagtatgtttcttccacat

SEQ ID NO: 69 - DNA, 24 bp, synthetic construct
  source 1..24: mol_type = other DNA
tgtgaaagtatgtttcttccacgt

SEQ ID NO: 70 - DNA, 25 bp, synthetic construct
  source 1..25: mol_type = other DNA
ttgtgaaagtatgtttcttccacgt

SEQ ID NO: 71 - DNA, 26 bp, synthetic construct
  source 1..26: mol_type = other DNA
attgtgaaagtatgtttcttccacgt

SEQ ID NO: 72 - DNA, 24 bp, synthetic construct
  source 1..24: mol_type = other DNA
cgtgctggcctcccacccccaccc

SEQ ID NO: 73 - DNA, 24 bp, synthetic construct
  source 1..24: mol_type = other DNA
cgtgctggcctcccacccccactc

SEQ ID NO: 74 - DNA, 24 bp, synthetic construct
  source 1..24: mol_type = other DNA
acatttaaaaagttcagatgttaa

SEQ ID NO: 75 - DNA, 24 bp, synthetic construct
  source 1..24: mol_type = other DNA
tctcatacttaactggttggtgat

SEQ ID NO: 76 - DNA, 22 bp, synthetic construct
  source 1..22: mol_type = other DNA
tattttccttacagggttccag

SEQ ID NO: 77 - DNA, 26 bp, synthetic construct
  source 1..26: mol_type = other DNA
gctggcagacttactccttaatttaa

SEQ ID NO: 78 - DNA, 29 bp, synthetic construct
  source 1..29: mol_type = other DNA
ataaagctatctatatatagctatctatg

SEQ ID NO: 79 - DNA, 21 bp, synthetic construct
  source 1..21: mol_type = other DNA
ccttctttttgattttgtctg

SEQ ID NO: 80 - DNA, 22 bp, synthetic construct
  source 1..22: mol_type = other DNA
tttattttccttacagggtttc

SEQ ID NO: 81 - DNA, 24 bp, synthetic construct
  source 1..24: mol_type = other DNA
gtgaaagtatgtttcttccacgta